European Patent Specification EP 3 801 561 B1, published March 19, 2025. Title: Methods for the Treatment of Bladder Cancer. Applicant: Eisai R&D Management Co., Ltd. Kim, Dae-Shik. The sequence listing filed with the application follows.

SEQUENCE LISTING (7 sequences)

SEQ ID NO: 1 - DNA, 1140 bp, Homo sapiens
atgccccactccagcctgcatccatccatcccgtgtcccaggggtcacggggcccagaaggcagccttggttctgctgagtgcctgcctggtgaccctttgggggctaggagagccaccagagcacactctccggtacctggtgctccacctagcctccctgcagctgggactgctgttaaacggggtctgcagcctggctgaggagctgcgccacatccactccaggtaccggggcagctactggaggactgtgcgggcctgcctgggctgccccctccgccgtggggccctgttgctgctgtccatctatttctactactccctcccaaatgcggtcggcccgcccttcacttggatgcttgccctcctgggcctctcgcaggcactgaacatcctcctgggcctcaagggcctggccccagctgagatctctgcagtgtgtgaaaaagggaatttcaacgtggcccatgggctggcatggtcatattacatcggatatctgcggctgatcctgccagagctccaggcccggattcgaacttacaatcagcattacaacaacctgctacggggtgcagtgagccagcggctgtatattctcctcccattggactgtggggtgcctgataacctgagtatggctgaccccaacattcgcttcctggataaactgccccagcagaccggtgaccgggctggcatcaaggatcgggtttacagcaacagcatctatgagcttctggagaacgggcagcgggcgggcacctgtgtcctggagtacgccacccccttgcagactttgtttgccatgtcacaatacagtcaagctggctttagccgggaggataggcttgagcaggccaaactcttctgccggacacttgaggacatcctggcagatgcccctgagtctcagaacaactgccgcctcattgcctaccaggaacctgcagatgacagcagcttctcgctgtcccaggaggttctccggcacctgcggcaggaggaaaaggaagaggttactgtgggcagcttgaagacctcagcggtgcccagtacctccacgatgtcccaagagcctgagctcctcatcagtggaatggaaaagcccctccctctccgcacggatttctcttga

SEQ ID NO: 2 - DNA, 1140 bp, Homo sapiens
atgccccactccagcctgcatccatccatcccgtgtcccaggggtcacggggcccagaaggcagccttggttctgctgagtgcctgcctggtgaccctttgggggctaggagagccaccagagcacactctccggtacctggtgctccacctagcctccctgcagctgggactgctgttaaacggggtctgcagcctggctgaggagctgcgccacatccactccaggtaccggggcagctactggaggactgtgcgggcctgcctgggctgccccctccgccgtggggccctgttgctgctgtccatctatttctactactccctcccaaatgcggtcggcccgcccttcacttggatgcttgccctcctgggcctctcgcaggcactgaacatcctcctgggcctcaagggcctggccccagctgagatctctgcagtgtgtgaaaaagggaatttcaacgtggcccatgggctggcatggtcatattacatcggatatctgcggctgatcctgccagagctccaggcccggattcgaacttacaatcagcattacaacaacctgctacggggtgcagtgagccagcggctgtatattctcctcccattggactgtggggtgcctgataacctgagtatggctgaccccaacattcgcttcctggataaactgccccagcagaccggtgaccatgctggcatcaaggatcgggtttacagcaacagcatctatgagcttctggagaacgggcagcgggcgggcacctgtgtcctggagtacgccacccccttgcagactttgtttgccatgtcacaatacagtcaagctggctttagccgggaggataggcttgagcaggccaaactcttctgccggacacttgaggacatcctggcagatgcccctgagtctcagaacaactgccgcctcattgcctaccaggaacctgcagatgacagcagcttctcgctgtcccaggaggttctccggcacctgcggcaggaggaaaaggaagaggttactgtgggcagcttgaagacctcagcggtgcccagtacctccacgatgtcccaagagcctgagctcctcatcagtggaatggaaaagcccctccctctccgcacggatttctcttga

SEQ ID NO: 3 - DNA, 1140 bp, Homo sapiens
atgccccactccagcctgcatccatccatcccgtgtcccaggggtcacggggcccagaaggcagccttggttctgctgagtgcctgcctggtgaccctttgggggctaggagagccaccagagcacactctccggtacctggtgctccacctagcctccctgcagctgggactgctgttaaacggggtctgcagcctggctgaggagctgcgccacatccactccaggtaccggggcagctactggaggactgtgcgggcctgcctgggctgccccctccgccgtggggccctgttgctgctgtccatctatttctactactccctcccaaatgcggtcggcccgcccttcacttggatgcttgccctcctgggcctctcgcaggcactgaacatcctcctgggcctcaagggcctggccccagctgagatctctgcagtgtgtgaaaaagggaatttcaacgtggcccatgggctggcatggtcatattacatcggatatctgcggctgatcctgccagagctccaggcccggattcgaacttacaatcagcattacaacaacctgctacggggtgcagtgagccagcggctgtatattctcctcccattggactgtggggtgcctgataacctgagtatggctgaccccaacattcgcttcctggataaactgccccagcagaccgctgaccgagctggcatcaaggatcgggtttacagcaacagcatctatgagcttctggagaacgggcagcgggcgggcacctgtgtcctggagtacgccacccccttgcagactttgtttgccatgtcacaatacagtcaagctggctttagccgggaggataggcttgagcaggccaaactcttctgccagacacttgaggacatcctggcagatgcccctgagtctcagaacaactgccgcctcattgcctaccaggaacctgcagatgacagcagcttctcgctgtcccaggaggttctccggcacctgcggcaggaggaaaaggaagaggttactgtgggcagcttgaagacctcagcggtgcccagtacctccacgatgtcccaagagcctgagctcctcatcagtggaatggaaaagcccctccctctccgcacggatttctcttga

SEQ ID NO: 4 - protein, 187 aa, Homo sapiens
VAHGLAWSYYIGYLRLILPELQARIRTYNQHYNNLLRGAVSQRLYILLPLDCGVPDNLSMADPNIRFLDKLPQQTGDRAGIKDRVYSNSIYELLENGQRAGTCVLEYATPLQTLFAMSQYSQAGFSREDRLEQAKLFCRTLEDILADAPESQNNCRLIAYQEPADDSSFSLSQEVLRHLRQEEKEEV

SEQ ID NO: 5 - protein, 311 aa, Artificial Sequence
  His-TEV-Sumo-WT STING construct
MHHHHHHSSGVDLGTENLYFQSNAMSDSEVNQEAKPEVKPEVKPETHINLKVSDGSSEIFFKIKKTTPLRRLMEAFAKRQGKEMDSLRFLYDGIRIQADQTPEDLDMEDNDIIEAHREQIGGGSVAHGLAWSYYIGYLRLILPELQARIRTYNQHYNNLLRGAVSQRLYILLPLDCGVPDNLSMADPNIRFLDKLPQQTGDRAGIKDRVYSNSIYELLENGQRAGTCVLEYATPLQTLFAMSQYSQAGFSREDRLEQAKLFCRTLEDILADAPESQNNCRLIAYQEPADDSSFSLSQEVLRHLRQEEKEEV

SEQ ID NO: 6 - protein, 187 aa, Homo sapiens
VAHGLAWSYYIGYLRLILPELQARIRTYNQHYNNLLRGAVSQRLYILLPLDCGVPDNLSMADPNIRFLDKLPQQTGDHAGIKDRVYSNSIYELLENGQRAGTCVLEYATPLQTLFAMSQYSQAGFSREDRLEQAKLFCRTLEDILADAPESQNNCRLIAYQEPADDSSFSLSQEVLRHLRQEEKEEV

SEQ ID NO: 7 - protein, 311 aa, Artificial Sequence
  His-TEV-Sumo-REF STING 155-341 construct
MHHHHHHSSGVDLGTENLYFQSNAMSDSEVNQEAKPEVKPEVKPETHINLKVSDGSSEIFFKIKKTTPLRRLMEAFAKRQGKEMDSLRFLYDGIRIQADQTPEDLDMEDNDIIEAHREQIGGGSVAHGLAWSYYIGYLRLILPELQARIRTYNQHYNNLLRGAVSQRLYILLPLDCGVPDNLSMADPNIRFLDKLPQQTGDHAGIKDRVYSNSIYELLENGQRAGTCVLEYATPLQTLFAMSQYSQAGFSREDRLEQAKLFCRTLEDILADAPESQNNCRLIAYQEPADDSSFSLSQEVLRHLRQEEKEEV